European Patent Application EP 4 219 558 A1, published August 2, 2023. Title: ANTIBODIES BINDING HUMAN CLAUDIN 18.2 AND USES THEREOF. Applicant: Beijing Mabworks Biotech Co., Ltd. The sequence listing filed with the application follows.

SEQUENCE LISTING (91 sequences)

SEQ ID NO: 1 - protein, 5 aa, synthetic construct
  REGION 1..5: note = HV-CDR1
SFWVN

SEQ ID NO: 2 - protein, 5 aa, synthetic construct
  REGION 1..5: note = HV-CDR1
SFWLN

SEQ ID NO: 3 - protein, 5 aa, synthetic construct
  REGION 1..5: note = HV-CDR3
SFWIN

SEQ ID NO: 4 - protein, 17 aa, synthetic construct
  REGION 1..17: note = HV-CDR2
NIYPSTSYTVYNQKFKD

SEQ ID NO: 5 - protein, 17 aa, synthetic construct
  REGION 1..17: note = HV-CDR2
NIYPSTSYTIYNQKFKD

SEQ ID NO: 6 - protein, 17 aa, synthetic construct
  REGION 1..17: note = HV-CDR2
NIYPSASYTVYNQKFKD

SEQ ID NO: 7 - protein, 9 aa, synthetic construct
  REGION 1..9: note = HV-CDR3
SWRGNSFDH

SEQ ID NO: 8 - protein, 9 aa, synthetic construct
  REGION 1..9: note = HV-CDR3
TWRGNSFDL

SEQ ID NO: 9 - protein, 9 aa, synthetic construct
  REGION 1..9: note = HV-CDR3
TWRGNSFDY

SEQ ID NO: 10 - protein, 17 aa, synthetic construct
  REGION 1..17: note = LV-CDR1
KSSQSLLNSGNQKNYVT

SEQ ID NO: 11 - protein, 17 aa, synthetic construct
  REGION 1..17: note = LV-CDR2
KSNQSLLNSGNQKNYVT

SEQ ID NO: 12 - protein, 17 aa, synthetic construct
  REGION 1..17: note = LV-CDR1
KSSQSLLNSGNQKNYLT

SEQ ID NO: 13 - protein, 7 aa, synthetic construct
  REGION 1..7: note = LV-CDR2
WGSTRVR

SEQ ID NO: 14 - protein, 7 aa, synthetic construct
  REGION 1..7: note = LV-CDR2
WGSTRST

SEQ ID NO: 15 - protein, 7 aa, synthetic construct
  REGION 1..7: note = LV-CDR2
WSSTRSF

SEQ ID NO: 16 - protein, 9 aa, synthetic construct
  REGION 1..9: note = LV-CDR3
QNDYTYPFT

SEQ ID NO: 17 - protein, 118 aa, synthetic construct
  REGION 1..118: note = HV
QVQLQQPGAELVRPGASVKLSCKASGYTFTSFWVNWVKQRPGQGLEWIGNIYPSTSYTVYNQKFKDKATLTVDKSSSTAYMQLSSPTSEDSAVYYCTRSWRGNSFDHWGQGTTLTVSS

SEQ ID NO: 18 - protein, 118 aa, synthetic construct
  REGION 1..118: note = HV
QVQLQQPGAELVRPGASVKLSCKASGYTFTSFWLNWVKQRPGQGLEWIGNIYPSTSYTVYNQKFKDKATLTVDKSSSTAYMQLSSPTSEDSAVYYCTRTWRGNSFDLWGQGTTLTVSS

SEQ ID NO: 19 - protein, 118 aa, synthetic construct
  REGION 1..118: note = HV
QVQLQQPGAELVRPGASVKLSCKASGYTFTSFWLNWVKQRPGQGLEWIGNIYPSTSYTVYNQKFKDKATLTVDKSSSTAYMQLSSPTSEDSAVYYCTRTWRGNSFDYWGQGTTLTVSS

SEQ ID NO: 20 - protein, 118 aa, synthetic construct
  REGION 1..118: note = HV
QVQLQQPGAELVRPGASVKLSCKASGYTFTSFWLNWVKQRPGQGLEWIGNIYPSTSYTIYNQKFKDKATLTVDKSSSTAYMQLSSPTSEDSAVYYCTRTWRGNSFDYWGQGTTLTVSS

SEQ ID NO: 21 - protein, 118 aa, synthetic construct
  REGION 1..118: note = HV
QVQLQQPGAELVRPGASVKLSCKASGYTFTSFWINWVKQRPGQGLEWIGNIYPSASYTVYNQKFKDKATLTVDKSSSTAYMQLSSPTSEDSAVYYCTRTWRGNSFDLWGQGTTLTVSS

SEQ ID NO: 22 - protein, 118 aa, synthetic construct
  REGION 1..118: note = HV
QVQLVQSGAEVKKPGASVKVSCKASGYTFTSFWLNWVRQAPGQGLEWMGNIYPSTSYTVYNQKFKDRVTMTRDTSTSTVYMELSSLRSEDTAVYYCARTWRGNSFDLWGQGTTVTVSS

SEQ ID NO: 23 - protein, 118 aa, synthetic construct
  REGION 1..118: note = HV
QVQLVQSGAEVKKPGASVKVSCKASGYTFTSFWLNWVRQAPGQGLEWIGNIYPSTSYTVYNQKFKDRVTLTVDKSTSTVYMELSSLRSEDTAVYYCARTWRGNSFDLWGQGTTVTVSS

SEQ ID NO: 24 - protein, 118 aa, synthetic construct
  REGION 1..118: note = HV
QVQLVQSGAEVKKPGASVKVSCKASGYTFTSFWLNWVRQAPGQGLEWIGNIYPSTSYTVYNQKFKDRVTLTVDTSTSTVYMELSSLRSEDTAVYYCARTWRGNSFDLWGQGTTVTVSS

SEQ ID NO: 25 - protein, 118 aa, synthetic construct
  REGION 1..118: note = HV
QVQLVQSGAEVKKPGASVKVSCKASGYTFTSFWLNWVRQRPGQGLEWIGNIYPSTSYTVYNQKFKDRVTLTVDKSTSTVYMELSSLRSEDTAVYYCARTWRGNSFDLWGQGTTVTVSS

SEQ ID NO: 26 - protein, 118 aa, synthetic construct
  REGION 1..118: note = HV
QVQLVQSGAEVKKPGASVKVSCKASGYTFTSFWLNWVRQRPGQGLEWIGNIYPSTSYTVYNQKFKDRVTLTVDKSTSTAYMELSSLRSEDTAVYYCTRTWRGNSFDLWGQGTTVTVSS

SEQ ID NO: 27 - protein, 118 aa, synthetic construct
  REGION 1..118: note = HV
QVQLVQSGAEVKKPGASVKVSCKASGYTFTSFWLNWVRQRPGQGLEWIGNIYPSTSYTVYNQKFKDRVTLTVDKSSSTAYMELSSLTSEDTAVYYCTRTWRGNSFDLWGQGTTVTVSS

SEQ ID NO: 28 - protein, 118 aa, synthetic construct
  REGION 1..118: note = HV
QVQLVQSGAEVKKPGASVKVSCKASGYTFTSFWLNWVKQRPGQGLEWIGNIYPSTSYTVYNQKFKDKVTLTVDKSTSTAYMELSSLRSEDTAVYYCTRTWRGNSFDLWGQGTTVTVSS

SEQ ID NO: 29 - protein, 118 aa, synthetic construct
  REGION 1..118: note = HV
QVQLVQSGAEVKKPGASVKVSCKASGYTFTSFWLNWVRQAPGQGLEWMGNIYPSTSYTVYNQKFKDRVTMTRDTSTSTVYMELSSLRSEDTAVYYCARTWRGNSFDYWGQGTTVTVSS

SEQ ID NO: 30 - protein, 118 aa, synthetic construct
  REGION 1..118: note = HV
QVQLVQSGAEVKKPGASVKVSCKASGYTFTSFWLNWVRQAPGQGLEWIGNIYPSTSYTVYNQKFKDRVTLTVDKSTSTVYMELSSLRSEDTAVYYCARTWRGNSFDYWGQGTTVTVSS

SEQ ID NO: 31 - protein, 118 aa, synthetic construct
  REGION 1..118: note = HV
QVQLVQSGAEVKKPGASVKVSCKASGYTFTSFWLNWVRQAPGQGLEWIGNIYPSTSYTVYNQKFKDRVTLTVDTSTSTVYMELSSLRSEDTAVYYCARTWRGNSFDYWGQGTTVTVSS

SEQ ID NO: 32 - protein, 118 aa, synthetic construct
  REGION 1..118: note = HV
QVQLVQSGAEVKKPGASVKVSCKASGYTFTSFWLNWVRQRPGQGLEWIGNIYPSTSYTVYNQKFKDRVTLTVDKSTSTVYMELSSLRSEDTAVYYCARTWRGNSFDYWGQGTTVTVSS

SEQ ID NO: 33 - protein, 118 aa, synthetic construct
  REGION 1..118: note = HV
QVQLVQSGAEVKKPGASVKVSCKASGYTFTSFWLNWVRQRPGQGLEWIGNIYPSTSYTVYNQKFKDRVTLTVDKSTSTAYMELSSLRSEDTAVYYCTRTWRGNSFDYWGQGTTVTVSS

SEQ ID NO: 34 - protein, 118 aa, synthetic construct
  REGION 1..118: note = HV
QVQLVQSGAEVKKPGASVKVSCKASGYTFTSFWLNWVRQRPGQGLEWIGNIYPSTSYTVYNQKFKDRVTLTVDKSSSTAYMELSSLTSEDTAVYYCTRTWRGNSFDYWGQGTTVTVSS

SEQ ID NO: 35 - protein, 118 aa, synthetic construct
  REGION 1..118: note = HV
QVQLVQSGAEVKKPGASVKVSCKASGYTFTSFWLNWVKQRPGQGLEWIGNIYPSTSYTVYNQKFKDKVTLTVDKSTSTAYMELSSLRSEDTAVYYCTRTWRGNSFDYWGQGTTVTVSS

SEQ ID NO: 36 - protein, 118 aa, synthetic construct
  REGION 1..118: note = HV
QVQLVQSGAEVKKPGASVKVSCKASGYTFTSFWLNWVRQAPGQGLEWMGNIYPSTSYTIYNQKFKDRVTMTRDTSTSTVYMELSSLRSEDTAVYYCARTWRGNSFDYWGQGTTVTVSS

SEQ ID NO: 37 - protein, 118 aa, synthetic construct
  REGION 1..118: note = HV
QVQLVQSGAEVKKPGASVKVSCKASGYTFTSFWLNWVRQAPGQGLEWIGNIYPSTSYTIYNQKFKDRVTLTVDKSTSTVYMELSSLRSEDTAVYYCARTWRGNSFDYWGQGTTVTVSS

SEQ ID NO: 38 - protein, 118 aa, synthetic construct
  REGION 1..118: note = HV
QVQLVQSGAEVKKPGASVKVSCKASGYTFTSFWLNWVRQAPGQGLEWIGNIYPSTSYTIYNQKFKDRVTLTVDTSTSTVYMELSSLRSEDTAVYYCARTWRGNSFDYWGQGTTVTVSS

SEQ ID NO: 39 - protein, 118 aa, synthetic construct
  REGION 1..118: note = HV
QVQLVQSGAEVKKPGASVKVSCKASGYTFTSFWLNWVRQRPGQGLEWIGNIYPSTSYTIYNQKFKDRVTLTVDKSTSTVYMELSSLRSEDTAVYYCARTWRGNSFDYWGQGTTVTVSS

SEQ ID NO: 40 - protein, 118 aa, synthetic construct
  REGION 1..118: note = HV
QVQLVQSGAEVKKPGASVKVSCKASGYTFTSFWLNWVRQRPGQGLEWIGNIYPSTSYTIYNQKFKDRVTLTVDKSTSTAYMELSSLRSEDTAVYYCTRTWRGNSFDYWGQGTTVTVSS

SEQ ID NO: 41 - protein, 118 aa, synthetic construct
  REGION 1..118: note = HV
QVQLVQSGAEVKKPGASVKVSCKASGYTFTSFWLNWVRQRPGQGLEWIGNIYPSTSYTIYNQKFKDRVTLTVDKSSSTAYMELSSLTSEDTAVYYCTRTWRGNSFDYWGQGTTVTVSS

SEQ ID NO: 42 - protein, 118 aa, synthetic construct
  REGION 1..118: note = HV
QVQLVQSGAEVKKPGASVKVSCKASGYTFTSFWLNWVKQRPGQGLEWIGNIYPSTSYTIYNQKFKDKVTLTVDKSTSTAYMELSSLRSEDTAVYYCTRTWRGNSFDYWGQGTTVTVSS

SEQ ID NO: 43 - protein, 118 aa, synthetic construct
  REGION 1..118: note = HV
QVQLVQSGAEVKKPGASVKVSCKASGYTFTSFWINWVRQAPGQGLEWMGNIYPSASYTVYNQKFKDRVTMTRDTSTSTVYMELSSLRSEDTAVYYCARTWRGNSFDLWGQGTTVTVSS

SEQ ID NO: 44 - protein, 118 aa, synthetic construct
  REGION 1..118: note = HV
QVQLVQSGAEVKKPGASVKVSCKASGYTFTSFWINWVRQAPGQGLEWIGNIYPSASYTVYNQKFKDRVTLTVDKSTSTVYMELSSLRSEDTAVYYCARTWRGNSFDLWGQGTTVTVSS

SEQ ID NO: 45 - protein, 118 aa, synthetic construct
  REGION 1..118: note = HV
QVQLVQSGAEVKKPGASVKVSCKASGYTFTSFWINWVRQAPGQGLEWIGNIYPSASYTVYNQKFKDRVTLTVDTSTSTVYMELSSLRSEDTAVYYCARTWRGNSFDLWGQGTTVTVSS

SEQ ID NO: 46 - protein, 118 aa, synthetic construct
  REGION 1..118: note = HV
QVQLVQSGAEVKKPGASVKVSCKASGYTFTSFWINWVRQRPGQGLEWIGNIYPSASYTVYNQKFKDRVTLTVDKSTSTVYMELSSLRSEDTAVYYCARTWRGNSFDLWGQGTTVTVSS

SEQ ID NO: 47 - protein, 118 aa, synthetic construct
  REGION 1..118: note = HV
QVQLVQSGAEVKKPGASVKVSCKASGYTFTSFWINWVRQRPGQGLEWIGNIYPSASYTVYNQKFKDRVTLTVDKSTSTAYMELSSLRSEDTAVYYCTRTWRGNSFDLWGQGTTVTVSS

SEQ ID NO: 48 - protein, 118 aa, synthetic construct
  REGION 1..118: note = HV
QVQLVQSGAEVKKPGASVKVSCKASGYTFTSFWINWVRQRPGQGLEWIGNIYPSASYTVYNQKFKDRVTLTVDKSSSTAYMELSSLTSEDTAVYYCTRTWRGNSFDLWGQGTTVTVSS

SEQ ID NO: 49 - protein, 118 aa, synthetic construct
  REGION 1..118: note = HV
QVQLVQSGAEVKKPGASVKVSCKASGYTFTSFWINWVKQRPGQGLEWIGNIYPSASYTVYNQKFKDKVTLTVDKSTSTAYMELSSLRSEDTAVYYCTRTWRGNSFDLWGQGTTVTVSS

SEQ ID NO: 50 - protein, 113 aa, synthetic construct
  REGION 1..113: note = LV
DIVMTQSPSSLTVTAGEKVTMSCKSSQSLLNSGNQKNYVTWYQQKPGQPPKLLIYWGSTRVRGVPDRFTGSGSGTDFTLTISSVQAEDLAVYYCQNDYTYPFTFGSGTKLEIK

SEQ ID NO: 51 - protein, 113 aa, synthetic construct
  REGION 1..113: note = LV
DIVMTQSPSSLTVTAGEKVTMSCKSNQSLLNSGNQKNYVTWYQQKPGQPPKLLIYWGSTRVRGVPDRFTGSGSGTDFTLTISSVQAEDLAVYYCQNDYTYPFTFGSGTKLEIK

SEQ ID NO: 52 - protein, 113 aa, synthetic construct
  REGION 1..113: note = LV
DIVMTQSPSSLTVTAGEKVTMSCKSSQSLLNSGNQKNYVTWYQQKPGQPPKLLIYWGSTRSTGVPDRFTGSGSGTDFTLTISSVQAEDLAVYYCQNDYTYPFTFGSGTKLEIK

SEQ ID NO: 53 - protein, 113 aa, synthetic construct
  REGION 1..113: note = LV
DIVMTQSPSSLTVTAGEKVTMSCKSSQSLLNSGNQKNYLTWYQQKPGQPPKLLIYWGSTRVRGVPDRFTGSGSGTDFTLTISSVQAEDLAVYYCQNDYTYPFTFGSGTKLEIK

SEQ ID NO: 54 - protein, 113 aa, synthetic construct
  REGION 1..113: note = LV
DIVMTQSPSSLTVTAGEKVTMSCKSSQSLLNSGNQKNYVTWYQQKPGQPPKLLIYWSSTRSFGVPDRFTGSGSGTDFTLTISSVQAEDLAVYYCQNDYTYPFTFGSGTKLEIK

SEQ ID NO: 55 - protein, 113 aa, synthetic construct
  REGION 1..113: note = LV
DIVMTQSPDSLAVSLGERATINCKSNQSLLNSGNQKNYVTWYQQKPGQPPKLLIYWGSTRVRGVPDRFSGSGSGTDFTLTISSLQAEDVAVYYCQNDYTYPFTFGQGTKLEIK

SEQ ID NO: 56 - protein, 113 aa, synthetic construct
  REGION 1..113: note = LV
DIVMTQSPSSLTVSLGEKATINCKSNQSLLNSGNQKNYVTWYQQKPGQPPKLLIYWGSTRVRGVPDRFSGSGSGTDFTLTISSLQAEDLAVYYCQNDYTYPFTFGQGTKLEIK

SEQ ID NO: 57 - protein, 113 aa, synthetic construct
  REGION 1..113: note = LV
DIVMTQSPSSLTVSLGEKATISCKSNQSLLNSGNQKNYVTWYQQKPGQPPKLLIYWGSTRVRGVPDRFSGSGSGTDFTLTISSLQAEDLAVYYCQNDYTYPFTFGSGTKLEIK

SEQ ID NO: 58 - protein, 113 aa, synthetic construct
  REGION 1..113: note = LV
DIVMTQSPDSLAVSLGERATINCKSSQSLLNSGNQKNYVTWYQQKPGQPPKLLIYWGSTRSTGVPDRFSGSGSGTDFTLTISSLQAEDVAVYYCQNDYTYPFTFGQGTKLEIK

SEQ ID NO: 59 - protein, 113 aa, synthetic construct
  REGION 1..113: note = LV
DIVMTQSPSSLTVSLGEKATINCKSSQSLLNSGNQKNYVTWYQQKPGQPPKLLIYWGSTRSTGVPDRFSGSGSGTDFTLTISSLQAEDLAVYYCQNDYTYPFTFGQGTKLEIK

SEQ ID NO: 60 - protein, 113 aa, synthetic construct
  REGION 1..113: note = LV
DIVMTQSPSSLTVSLGEKATISCKSSQSLLNSGNQKNYVTWYQQKPGQPPKLLIYWGSTRSTGVPDRFSGSGSGTDFTLTISSLQAEDLAVYYCQNDYTYPFTFGSGTKLEIK

SEQ ID NO: 61 - protein, 113 aa, synthetic construct
  REGION 1..113: note = LV
DIVMTQSPDSLAVSLGERATINCKSSQSLLNSGNQKNYLTWYQQKPGQPPKLLIYWGSTRVRGVPDRFSGSGSGTDFTLTISSLQAEDVAVYYCQNDYTYPFTFGQGTKLEIK

SEQ ID NO: 62 - protein, 113 aa, synthetic construct
  REGION 1..113: note = LV
DIVMTQSPSSLTVSLGEKATINCKSSQSLLNSGNQKNYLTWYQQKPGQPPKLLIYWGSTRVRGVPDRFSGSGSGTDFTLTISSLQAEDLAVYYCQNDYTYPFTFGQGTKLEIK

SEQ ID NO: 63 - protein, 113 aa, synthetic construct
  REGION 1..113: note = LV
DIVMTQSPSSLTVSLGEKATISCKSSQSLLNSGNQKNYLTWYQQKPGQPPKLLIYWGSTRVRGVPDRFSGSGSGTDFTLTISSLQAEDLAVYYCQNDYTYPFTFGSGTKLEIK

SEQ ID NO: 64 - protein, 113 aa, synthetic construct
  REGION 1..113: note = LV
DIVMTQSPDSLAVSLGERATINCKSSQSLLNSGNQKNYVTWYQQKPGQPPKLLIYWSSTRSFGVPDRFSGSGSGTDFTLTISSLQAEDVAVYYCQNDYTYPFTFGQGTKLEIK

SEQ ID NO: 65 - protein, 113 aa, synthetic construct
  REGION 1..113: note = LV
DIVMTQSPSSLTVSLGEKATINCKSSQSLLNSGNQKNYVTWYQQKPGQPPKLLIYWSSTRSFGVPDRFSGSGSGTDFTLTISSLQAEDLAVYYCQNDYTYPFTFGQGTKLEIK

SEQ ID NO: 66 - protein, 113 aa, synthetic construct
  REGION 1..113: note = LV
DIVMTQSPSSLTVSLGEKATISCKSSQSLLNSGNQKNYVTWYQQKPGQPPKLLIYWSSTRSFGVPDRFSGSGSGTDFTLTISSLQAEDLAVYYCQNDYTYPFTFGSGTKLEIK

SEQ ID NO: 67 - protein, 330 aa, synthetic construct [sequence omitted]

SEQ ID NO: 68 - protein, 107 aa, synthetic construct [sequence omitted]

SEQ ID NO: 69 - DNA, 786 bp, Homo sapiens
  source 1..786: mol_type = other DNA
atgagcaccaccacctgccaggtggtggccttcctgctgagcatcctgggcctggccggctgcatcgccgccaccggcatggacatgtggagcacccaggacctgtacgacaaccccgtgaccagcgtgttccagtacgagggcctgtggcgcagctgcgtgcgccagagcagcggcttcaccgagtgccgcccctacttcaccatcctgggcctgcccgccatgctgcaggccgtgcgcgccctgatgatcgtgggcatcgtgctgggcgccatcggcctgctggtgagcatcttcgccctgaagtgcatccgcatcggcagcatggaggacagcgccaaggccaacatgaccctgaccagcggcatcatgttcatcgtgagcggcctgtgcgccatcgccggcgtgagcgtgttcgccaacatgctggtgaccaacttctggatgagcaccgccaacatgtacaccggcatgggcggcatggtgcagaccgtgcagacccgctacaccttcggcgccgccctgttcgtgggctgggtggccggcggcctgaccctgatcggcggcgtgatgatgtgcatcgcctgccgcggcctggcccccgaggagaccaactacaaggccgtgagctaccacgccagcggccacagcgtggcctacaagcccggcggcttcaaggccagcaccggcttcggcagcaacaccaagaacaagaagatctacgacggcggcgcccgcaccgaggacgaggtgcagagctaccccagcaagcacgactacgtgtaa

SEQ ID NO: 70 - protein, 261 aa, Homo sapiens
MSTTTCQVVAFLLSILGLAGCIAATGMDMWSTQDLYDNPVTSVFQYEGLWRSCVRQSSGFTECRPYFTILGLPAMLQAVRALMIVGIVLGAIGLLVSIFALKCIRIGSMEDSAKANMTLTSGIMFIVSGLCAIAGVSVFANMLVTNFWMSTANMYTGMGGMVQTVQTRYTFGAALFVGWVAGGLTLIGGVMMCIACRGLAPEETNYKAVSYHASGHSVAYKPGGFKASTGFGSNTKNKKIYDGGARTEDEVQSYPSKHDYV

SEQ ID NO: 71 - DNA, 786 bp, Homo sapiens
  source 1..786: mol_type = other DNA
atggccgtgaccgcctgccagggcctgggcttcgtggtgagcctgatcggcatcgccggcatcatcgccgccacctgcatggaccagtggagcacccaggacctgtacaacaaccccgtgaccgccgtgttcaactaccagggcctgtggcgcagctgcgtgcgcgagagcagcggcttcaccgagtgccgcggctacttcaccctgctgggcctgcccgccatgctgcaggccgtgcgcgccctgatgatcgtgggcatcgtgctgggcgccatcggcctgctggtgagcatcttcgccctgaagtgcatccgcatcggcagcatggaggacagcgccaaggccaacatgaccctgaccagcggcatcatgttcatcgtgagcggcctgtgcgccatcgccggcgtgagcgtgttcgccaacatgctggtgaccaacttctggatgagcaccgccaacatgtacaccggcatgggcggcatggtgcagaccgtgcagacccgctacaccttcggcgccgccctgttcgtgggctgggtggccggcggcctgaccctgatcggcggcgtgatgatgtgcatcgcctgccgcggcctggcccccgaggagaccaactacaaggccgtgagctaccacgccagcggccacagcgtggcctacaagcccggcggcttcaaggccagcaccggcttcggcagcaacaccaagaacaagaagatctacgacggcggcgcccgcaccgaggacgaggtgcagagctaccccagcaagcacgactacgtgtaa

SEQ ID NO: 72 - protein, 261 aa, Homo sapiens
MAVTACQGLGFVVSLIGIAGIIAATCMDQWSTQDLYNNPVTAVFNYQGLWRSCVRESSGFTECRGYFTLLGLPAMLQAVRALMIVGIVLGAIGLLVSIFALKCIRIGSMEDSAKANMTLTSGIMFIVSGLCAIAGVSVFANMLVTNFWMSTANMYTGMGGMVQTVQTRYTFGAALFVGWVAGGLTLIGGVMMCIACRGLAPEETNYKAVSYHASGHSVAYKPGGFKASTGFGSNTKNKKIYDGGARTEDEVQSYPSKHDYV

SEQ ID NO: 73 - protein, 261 aa, synthetic construct
  REGION 1..261: note = Mutant 1
MAVTACQGLGFVVSLIGIAGIIAATCMDMWSTQDLYNNPVTAVFNYQGLWRSCVRESSGFTECRGYFTLLGLPAMLQAVRALMIVGIVLGAIGLLVSIFALKCIRIGSMEDSAKANMTLTSGIMFIVSGLCAIAGVSVFANMLVTNFWMSTANMYTGMGGMVQTVQTRYTFGAALFVGWVAGGLTLIGGVMMCIACRGLAPEETNYKAVSYHASGHSVAYKPGGFKASTGFGSNTKNKKIYDGGARTEDEVQSYPSKHDYV

SEQ ID NO: 74 - protein, 261 aa, synthetic construct
  REGION 1..261: note = Mutant 2
MAVTACQGLGFVVSLIGIAGIIAATCMDQWSTQDLYDNPVTAVFNYQGLWRSCVRESSGFTECRGYFTLLGLPAMLQAVRALMIVGIVLGAIGLLVSIFALKCIRIGSMEDSAKANMTLTSGIMFIVSGLCAIAGVSVFANMLVTNFWMSTANMYTGMGGMVQTVQTRYTFGAALFVGWVAGGLTLIGGVMMCIACRGLAPEETNYKAVSYHASGHSVAYKPGGFKASTGFGSNTKNKKIYDGGARTEDEVQSYPSKHDYV

SEQ ID NO: 75 - protein, 261 aa, synthetic construct
  REGION 1..261: note = Mutant 3
MAVTACQGLGFVVSLIGIAGIIAATCMDQWSTQDLYNNPVTSVFNYQGLWRSCVRESSGFTECRGYFTLLGLPAMLQAVRALMIVGIVLGAIGLLVSIFALKCIRIGSMEDSAKANMTLTSGIMFIVSGLCAIAGVSVFANMLVTNFWMSTANMYTGMGGMVQTVQTRYTFGAALFVGWVAGGLTLIGGVMMCIACRGLAPEETNYKAVSYHASGHSVAYKPGGFKASTGFGSNTKNKKIYDGGARTEDEVQSYPSKHDYV

SEQ ID NO: 76 - protein, 261 aa, synthetic construct
  REGION 1..261: note = Mutant 4
MAVTACQGLGFVVSLIGIAGIIAATCMDQWSTQDLYNNPVTAVFQYQGLWRSCVRESSGFTECRGYFTLLGLPAMLQAVRALMIVGIVLGAIGLLVSIFALKCIRIGSMEDSAKANMTLTSGIMFIVSGLCAIAGVSVFANMLVTNFWMSTANMYTGMGGMVQTVQTRYTFGAALFVGWVAGGLTLIGGVMMCIACRGLAPEETNYKAVSYHASGHSVAYKPGGFKASTGFGSNTKNKKIYDGGARTEDEVQSYPSKHDYV

SEQ ID NO: 77 - protein, 261 aa, synthetic construct
  REGION 1..261: note = Mutant 5
MAVTACQGLGFVVSLIGIAGIIAATCMDQWSTQDLYNNPVTAVFNYEGLWRSCVRESSGFTECRGYFTLLGLPAMLQAVRALMIVGIVLGAIGLLVSIFALKCIRIGSMEDSAKANMTLTSGIMFIVSGLCAIAGVSVFANMLVTNFWMSTANMYTGMGGMVQTVQTRYTFGAALFVGWVAGGLTLIGGVMMCIACRGLAPEETNYKAVSYHASGHSVAYKPGGFKASTGFGSNTKNKKIYDGGARTEDEVQSYPSKHDYV

SEQ ID NO: 78 - protein, 261 aa, synthetic construct
  REGION 1..261: note = Mutant 6
MAVTACQGLGFVVSLIGIAGIIAATCMDQWSTQDLYNNPVTAVFNYQGLWRSCVRQSSGFTECRGYFTLLGLPAMLQAVRALMIVGIVLGAIGLLVSIFALKCIRIGSMEDSAKANMTLTSGIMFIVSGLCAIAGVSVFANMLVTNFWMSTANMYTGMGGMVQTVQTRYTFGAALFVGWVAGGLTLIGGVMMCIACRGLAPEETNYKAVSYHASGHSVAYKPGGFKASTGFGSNTKNKKIYDGGARTEDEVQSYPSKHDYV

SEQ ID NO: 79 - protein, 261 aa, synthetic construct
  REGION 1..261: note = Mutant 7
MAVTACQGLGFVVSLIGIAGIIAATCMDQWSTQDLYNNPVTAVFNYQGLWRSCVRESSGFTECRPYFTLLGLPAMLQAVRALMIVGIVLGAIGLLVSIFALKCIRIGSMEDSAKANMTLTSGIMFIVSGLCAIAGVSVFANMLVTNFWMSTANMYTGMGGMVQTVQTRYTFGAALFVGWVAGGLTLIGGVMMCIACRGLAPEETNYKAVSYHASGHSVAYKPGGFKASTGFGSNTKNKKIYDGGARTEDEVQSYPSKHDYV

SEQ ID NO: 80 - protein, 261 aa, synthetic construct
  REGION 1..261: note = Mutant 8
MAVTACQGLGFVVSLIGIAGIIAATCMDQWSTQDLYNNPVTAVFNYQGLWRSCVRESSGFTECRGYFTILGLPAMLQAVRALMIVGIVLGAIGLLVSIFALKCIRIGSMEDSAKANMTLTSGIMFIVSGLCAIAGVSVFANMLVTNFWMSTANMYTGMGGMVQTVQTRYTFGAALFVGWVAGGLTLIGGVMMCIACRGLAPEETNYKAVSYHASGHSVAYKPGGFKASTGFGSNTKNKKIYDGGARTEDEVQSYPSKHDYV

SEQ ID NO: 81 - protein, 261 aa, synthetic construct
  REGION 1..261: note = Mutant 9
MAVTACQGLGFVVSLIGIAGIIAATCMDQWSTQDLYNNPVTSVFQYQGLWRSCVRESSGFTECRGYFTLLGLPAMLQAVRALMIVGIVLGAIGLLVSIFALKCIRIGSMEDSAKANMTLTSGIMFIVSGLCAIAGVSVFANMLVTNFWMSTANMYTGMGGMVQTVQTRYTFGAALFVGWVAGGLTLIGGVMMCIACRGLAPEETNYKAVSYHASGHSVAYKPGGFKASTGFGSNTKNKKIYDGGARTEDEVQSYPSKHDYV

SEQ ID NO: 82 - protein, 261 aa, synthetic construct
  REGION 1..261: note = Mutant 10
MAVTACQGLGFVVSLIGIAGIIAATCMDQWSTQDLYNNPVTSVFNYEGLWRSCVRESSGFTECRGYFTLLGLPAMLQAVRALMIVGIVLGAIGLLVSIFALKCIRIGSMEDSAKANMTLTSGIMFIVSGLCAIAGVSVFANMLVTNFWMSTANMYTGMGGMVQTVQTRYTFGAALFVGWVAGGLTLIGGVMMCIACRGLAPEETNYKAVSYHASGHSVAYKPGGFKASTGFGSNTKNKKIYDGGARTEDEVQSYPSKHDYV

SEQ ID NO: 83 - protein, 261 aa, synthetic construct
  REGION 1..261: note = Mutant 11
MAVTACQGLGFVVSLIGIAGIIAATCMDQWSTQDLYNNPVTAVFQYEGLWRSCVRESSGFTECRGYFTLLGLPAMLQAVRALMIVGIVLGAIGLLVSIFALKCIRIGSMEDSAKANMTLTSGIMFIVSGLCAIAGVSVFANMLVTNFWMSTANMYTGMGGMVQTVQTRYTFGAALFVGWVAGGLTLIGGVMMCIACRGLAPEETNYKAVSYHASGHSVAYKPGGFKASTGFGSNTKNKKIYDGGARTEDEVQSYPSKHDYV

SEQ ID NO: 84 - protein, 261 aa, synthetic construct
  REGION 1..261: note = Mutant 12
MAVTACQGLGFVVSLIGIAGIIAATCMDQWSTQDLYNNPVTSVFQYEGLWRSCVRESSGFTECRGYFTLLGLPAMLQAVRALMIVGIVLGAIGLLVSIFALKCIRIGSMEDSAKANMTLTSGIMFIVSGLCAIAGVSVFANMLVTNFWMSTANMYTGMGGMVQTVQTRYTFGAALFVGWVAGGLTLIGGVMMCIACRGLAPEETNYKAVSYHASGHSVAYKPGGFKASTGFGSNTKNKKIYDGGARTEDEVQSYPSKHDYV

SEQ ID NO: 85 - protein, 261 aa, synthetic construct
  REGION 1..261: note = Mutant 13
MAVTACQGLGFVVSLIGIAGIIAATCMDQWSTQDLYNNPVTSVFQYEGLWRSCVRQSSGFTECRGYFTLLGLPAMLQAVRALMIVGIVLGAIGLLVSIFALKCIRIGSMEDSAKANMTLTSGIMFIVSGLCAIAGVSVFANMLVTNFWMSTANMYTGMGGMVQTVQTRYTFGAALFVGWVAGGLTLIGGVMMCIACRGLAPEETNYKAVSYHASGHSVAYKPGGFKASTGFGSNTKNKKIYDGGARTEDEVQSYPSKHDYV

SEQ ID NO: 86 - protein, 261 aa, synthetic construct
  REGION 1..261: note = Mutant 14
MSTTTCQVVAFLLSILGLAGCIAATGMDMWSTQDLYDNPVTSVFQYEGLWRSCVRESSGFTECRPYFTILGLPAMLQAVRALMIVGIVLGAIGLLVSIFALKCIRIGSMEDSAKANMTLTSGIMFIVSGLCAIAGVSVFANMLVTNFWMSTANMYTGMGGMVQTVQTRYTFGAALFVGWVAGGLTLIGGVMMCIACRGLAPEETNYKAVSYHASGHSVAYKPGGFKASTGFGSNTKNKKIYDGGARTEDEVQSYPSKHDYV

SEQ ID NO: 87 - protein, 261 aa, synthetic construct
  REGION 1..261: note = Mutant 15
MSTTTCQVVAFLLSILGLAGCIAATGMDMWSTQDLYDNPVTAVFNYEGLWRSCVRESSGFTECRPYFTILGLPAMLQAVRALMIVGIVLGAIGLLVSIFALKCIRIGSMEDSAKANMTLTSGIMFIVSGLCAIAGVSVFANMLVTNFWMSTANMYTGMGGMVQTVQTRYTFGAALFVGWVAGGLTLIGGVMMCIACRGLAPEETNYKAVSYHASGHSVAYKPGGFKASTGFGSNTKNKKIYDGGARTEDEVQSYPSKHDYV

SEQ ID NO: 88 - protein, 261 aa, synthetic construct
  REGION 1..261: note = Mutant 16
MSTTTCQVVAFLLSILGLAGCIAATGMDMWSTQDLYDNPVTAVFNYQGLWRSCVRESSGFTECRPYFTILGLPAMLQAVRALMIVGIVLGAIGLLVSIFALKCIRIGSMEDSAKANMTLTSGIMFIVSGLCAIAGVSVFANMLVTNFWMSTANMYTGMGGMVQTVQTRYTFGAALFVGWVAGGLTLIGGVMMCIACRGLAPEETNYKAVSYHASGHSVAYKPGGFKASTGFGSNTKNKKIYDGGARTEDEVQSYPSKHDYV

SEQ ID NO: 89 - protein, 330 aa, synthetic construct
  REGION 1..330: note = Mouse IgG2a constant region
AKTTAPSVYPLAPVCGDTTGSSVTLGCLVKGYFPEPVTLTWNSGSLSSGVHTFPAVLQSDLYTLSSSVTVTSSTWPSQSITCNVAHPASSTKVDKKIEPRGPTIKPCPPCKCPAPNLLGGPSVFIFPPKIKDVLMISLSPIVTCVVVDVSEDDPDVQISWFVNNVEVHTAQTQTHREDYNSTLRVVSALPIQHQDWMSGKEFKCKVNNKDLPAPIERTISKPKGSVRAPQVYVLPPPEEEMTKKQVTLTCMVTDFMPEDIYVEWTNNGKTELNYKNTEPVLDSDGSYFMYSKLRVEKKNWVERNSYSCSVVHEGLHNHHTTKSFSRTPGK

SEQ ID NO: 90 - protein, 107 aa, synthetic construct
  REGION 1..107: note = Mouse kappa constant region
RADAAPTVSIFPPSSEQLTSGGASVVCFLNNFYPKDINVKWKIDGSERQNGVLNSWTDQDSKDSTYSMSSTLTLTKDEYERHNSYTCEATHKTSTSPIVKSFNRNEC

SEQ ID NO: 91 - protein, 5 aa, synthetic construct
  REGION 1..5: note = Peptide linker
PVGVV